European Patent Application EP 4 154 732 A1, published March 29, 2023. Title: Citrus-like flavor composition, citrus flavored beverage. Applicant: Takasago International Corporation. The sequence listing filed with the application follows.

SEQUENCE LISTING (4 sequences)

SEQ ID NO: 1 - DNA, 945 bp, Homo sapiens
  CDS (1)..(945)
atggctgaaaggaattacaccgtagtgacggagttcttccttactgcatttactgaacatctccagtggagggttcctctcttcctcatatttttgagtttctatcttgccactatgttagggaacacaggcatgatcctcctgatccgtggcgatcgtcggctccacaccccgatgtacttcttcctcagccacctttccttggtggacatctgctactcgtccgccatcatccctcagatgctggctgtgctgtgggagcacggcacaaccatctcccaggctcgctgtgcagctcagttcttcctcttcaccttctttgcctccatcgactgctaccttctggccatcatggcctatgaccgctacacggccgtgtgccagcccctgctttatgtcaccatcataaccgagaaggcccgctggggcctagtcactggggcttacgttgctggttttttcagtgcctttgttcgaacggtcacagccttcactctctccttttgtggaaacaatgagatcaacttcattttctgtgacctccctcctctattaaaactctcctgtggggacagctacactcaggaagtggtgattattgtgtttgctcttttcgtcatgcctgcctgtatcttggtgatcttggtatcctacctgtttatcattgtggccatcctgcagatccactctgctggaggccgggccaagaccttctccacctgcgcctcccacctcactgccgtcgctcttttctttggcaccctcatcttcatgtacctgcgagacaacacaggccagtcctccgagggagaccgagtggtgtctgtgctctacacggtggtgaccccaatgctgaatccccttatctatagcctgagaaacaaggaggtaaaagaggccactaggaaagccctgagcaaatcaaagcctgctagaagaccctaa

SEQ ID NO: 2 - protein, 314 aa, Homo sapiens
MAERNYTVVTEFFLTAFTEHLQWRVPLFLIFLSFYLATMLGNTGMILLIRGDRRLHTPMYFFLSHLSLVDICYSSAIIPQMLAVLWEHGTTISQARCAAQFFLFTFFASIDCYLLAIMAYDRYTAVCQPLLYVTIITEKARWGLVTGAYVAGFFSAFVRTVTAFTLSFCGNNEINFIFCDLPPLLKLSCGDSYTQEVVIIVFALFVMPACILVILVSYLFIIVAILQIHSAGGRAKTFSTCASHLTAVALFFGTLIFMYLRDNTGQSSEGDRVVSVLYTVVTPMLNPLIYSLRNKEVKEATRKALSKSKPARRP

SEQ ID NO: 3 - DNA, 1057 bp, Bos taurus
  CDS (1)..(1047)
atgaacgggaccgagggcccaaacttctacgtgcctttctccaacaagacgggcgtggtgcgcagccccttcgaggccccgcagtactacctggcggagccatggcagttctccatgctggccgcctacatgttcctgctgatcatgcttggcttccccatcaacttcctcacgctgtacgtcacagtccagcacaagaagctgcgcacacccctcaactacatcctgctcaacctggccgtggccgacctcttcatggtcttcgggggcttcaccaccaccctctacacctctctgcacggatacttcgtctttgggcccacgggctgcaacctggagggcttctttgccaccctgggcggtgaaattgcactgtggtccttggtggtcctggccatcgagcggtacgtggtggtgtgcaagcccatgagcaacttccgcttcggggagaaccacgccatcatgggcgtcgccttcacctgggtcatggctctggcctgtgccgcgccccccctcgtcggctggtccaggtacatcccggagggcatgcagtgctcgtgcgggattgactactacacgccccacgaggagaccaacaatgagtcgttcgtcatctacatgttcgtggtccacttcatcatccccctgattgtcatattcttctgctacgggcagctggtgttcaccgtcaaggaggcggctgcccagcagcaggagtcggccaccactcagaaggccgagaaggaggtcacccgcatggtgatcatcatggtcatcgctttcctaatctgctggctgccctacgctggggtggcgttctacatcttcacccatcagggctctgactttggccccatcttcatgaccatcccggctttctttgccaagacttctgccgtctacaaccccgtcatctacatcatgatgaacaagcagttccggaactgcatggtcaccactctctgctgtggcaagaacccgctgggtgacgacgaggcctccaccaccgtctccaagacagagaccagccaggtggcgcctgcctaagcccctccag

SEQ ID NO: 4 - protein, 348 aa, Bos taurus
MNGTEGPNFYVPFSNKTGVVRSPFEAPQYYLAEPWQFSMLAAYMFLLIMLGFPINFLTLYVTVQHKKLRTPLNYILLNLAVADLFMVFGGFTTTLYTSLHGYFVFGPTGCNLEGFFATLGGEIALWSLVVLAIERYVVVCKPMSNFRFGENHAIMGVAFTWVMALACAAPPLVGWSRYIPEGMQCSCGIDYYTPHEETNNESFVIYMFVVHFIIPLIVIFFCYGQLVFTVKEAAAQQQESATTQKAEKEVTRMVIIMVIAFLICWLPYAGVAFYIFTHQGSDFGPIFMTIPAFFAKTSAVYNPVIYIMMNKQFRNCMVTTLCCGKNPLGDDEASTTVSKTETSQVAPA